European Patent Specification EP 3 857 222 B1, published December 6, 2023. Title: High throughput epitope identification and T cell receptor specificity determination using loadable detection molecules. Applicant: Danmarks Tekniske Universitet (DTU) Reker Hadrup, Sine Nyboe Jakobsen, Søren Kumar Saini, Sunil. The sequence listing filed with the application follows.

SEQUENCE LISTING (43 sequences)

SEQ ID NO: 1 - protein, 275 aa, Homo sapiens [sequence omitted]

SEQ ID NO: 2 - protein, 274 aa, Homo sapiens
  Cys-mut HLA-A 0201 heavy chain w/o TM domain (1)..(1)
GSHSMRYFFTSVSRPGRGEPRFIAVGYVDDTQFVRFDSDAASQRMEPRAPWIEQEGPEYWDGETRKVKAHSQTHRVDLGTLRGCYNQSEAGSHTVQRMYGCDVGSDWRFLRGYHQYAYDGKDYIALKEDLRSWTAADMCAQTTKHKWEAAHVAEQLRAYLEGTCVEWLRRYLENGKETLQRTDAPKTHMTHHAVSDHEATLRCWALSFYPAEITLTWQRDGEDQTQDTELVETRPAGDGTFQKWAAVVVPSGQEQRYTCHVQHEGLPKPLTLRW

SEQ ID NO: 3 - protein, 274 aa, Homo sapiens
  Cys-mut HLA-A 0101 heavy chain w/o TM domain (1)..(1)
GSHSMRYFFTSVSRPGRGEPRFIAVGYVDDTQFVRFDSDAASQKMEPRAPWIEQEGPEYWDQETRNMKAHSQTDRANLGTLRGCYNQSEDGSHTIQIMYGCDVGPDGRFLRGYRQDAYDGKDYIALNEDLRSWTAADMCAQITKRKWEAVHAAEQRRVYLEGRCVDGLRRYLENGKETLQRTDPPKTHMTHHPISDHEATLRCWALGFYPAEITLTWQRDGEDQTQDTELVETRPAGDGTFQKWAAVVVPSGEEQRYTCHVQHEGLPKPLTLRW

SEQ ID NO: 4 - protein, 274 aa, Homo sapiens
  Cys-mut HLA-A 0301 heavy chain w/o TM domain (1)..(1)
GSHSMRYFFTSVSRPGRGEPRFIAVGYVDDTQFVRFDSDAASQRMEPRAPWIEQEGPEYWDQETRNVKAQSQTDRVDLGTLRGCYNQSEAGSHTIQIMYGCDVGSDGRFLRGYRQDAYDGKDYIALNEDLRSWTAADMCAQITKRKWEAAHEAEQLRAYLDGTCVEWLRRYLENGKETLQRTDPPKTHMTHHPISDHEATLRCWALGFYPAEITLTWQRDGEDQTQDTELVETRPAGDGTFQKWAAVVVPSGEEQRYTCHVQHEGLPKPLTLRW

SEQ ID NO: 5 - protein, 274 aa, Homo sapiens
  Cys-mut HLA-A 1101 heavy chain w/o TM domain (1)..(1)
GSHSMRYFYTSVSRPGRGEPRFIAVGYVDDTQFVRFDSDAASQRMEPRAPWIEQEGPEYWDQETRNVKAQSQTDRVDLGTLRGCYNQSEDGSHTIQIMYGCDVGPDGRFLRGYRQDAYDGKDYIALNEDLRSWTAADMCAQITKRKWEAAHAAEQQRAYLEGRCVEWLRRYLENGKETLQRTDPPKTHMTHHPISDHEATLRCWALGFYPAEITLTWQRDGEDQTQDTELVETRPAGDGTFQKWAAVVVPSGEEQRYTCHVQHEGLPKPLTLRW

SEQ ID NO: 6 - protein, 274 aa, Homo sapiens
  Cys-mut HLA-A 2402 heavy chain w/o TM domain (1)..(1)
GSHSMRYFSTSVSRPGRGEPRFIAVGYVDDTQFVRFDSDAASQRMEPRAPWIEQEGPEYWDEETGKVKAHSQTDRENLRIALRCYNQSEAGSHTLQMMFGCDVGSDGRFLRGYHQYAYDGKDYIALKEDLRSWTAADMCAQITKRKWEAAHVAEQQRAYLEGTCVDGLRRYLENGKETLQRTDPPKTHMTHHPISDHEATLRCWALGFYPAEITLTWQRDGEDQTQDTELVETRPAGDGTFQKWAAVVVPSGEEQRYTCHVQHEGLPKPLTLRW

SEQ ID NO: 7 - protein, 274 aa, Homo sapiens
  Cys-mut HLA-B 0702 heavy chain w/o TM domain (1)..(1)
GSHSMRYFYTSVSRPGRGEPRFISVGYVDDTQFVRFDSDAASPREEPRAPWIEQEGPEYWDRNTQIYKAQAQTDRESLRNLRGCYNQSEAGSHTLQSMYGCDVGPDGRLLRGHDQYAYDGKDYIALNEDLRSWTAADTCAQITQRKWEAAREAEQRRAYLEGECVEWLRRYLENGKDKLERADPPKTHVTHHPISDHEATLRCWALGFYPAEITLTWQRDGEDQTQDTELVETRPAGDRTFQKWAAVVVPSGEEQRYTCHVQHEGLPKPLTLRW

SEQ ID NO: 8 - protein, 274 aa, Homo sapiens
  Cys-mut HLA-B 0801 heavy chain w/o TM domain (1)..(1)
GSHSMRYFDTAMSRPGRGEPRFISVGYVDDTQFVRFDSDAASPREEPRAPWIEQEGPEYWDRNTQIFKTNTQTDRESLRNLRGCYNQSEAGSHTLQSMYGCDVGPDGRLLRGHNQYAYDGKDYIALNEDLRSWTAADTCAQITQRKWEAARVAEQDRAYLEGTCVEWLRRYLENGKDTLERADPPKTHVTHHPISDHEATLRCWALGFYPAEITLTWQRDGEDQTQDTELVETRPAGDRTFQKWAAVVVPSGEEQRYTCHVQHEGLPKPLTLRW

SEQ ID NO: 9 - protein, 274 aa, Homo sapiens
  Cys-mut HLA-B 1501 heavy chain w/o TM domain (1)..(1)
GSHSMRYFYTAMSRPGRGEPRFIAVGYVDDTQFVRFDSDAASPRMAPRAPWIEQEGPEYWDRETQISKTNTQTYRESLRNLRGCYNQSEAGSHTLQRMYGCDVGPDGRLLRGHDQSAYDGKDYIALNEDLSSWTAADTCAQITQRKWEAAREAEQWRAYLEGLCVEWLRRYLENGKETLQRADPPKTHVTHHPISDHEATLRCWALGFYPAEITLTWQRDGEDQTQDTELVETRPAGDRTFQKWAAVVVPSGEEQRYTCHVQHEGLPKPLTLRW

SEQ ID NO: 10 - protein, 274 aa, Homo sapiens
  Cys-mut HLA-B 3501 heavy chain w/o TM domain (1)..(1)
GSHSMRYFYTAMSRPGRGEPRFIAVGYVDDTQFVRFDSDAASPRTEPRAPWIEQEGPEYWDRNTQIFKTNTQTYRESLRNLRGCYNQSEAGSHIIQRMYGCDLGPDGRLLRGHDQSAYDGKDYIALNEDLSSWTAADTCAQITQRKWEAARVAEQLRAYLEGLCVEWLRRYLENGKETLQRADPPKTHVTHHPVSDHEATLRCWALGFYPAEITLTWQRDGEDQTQDTELVETRPAGDRTFQKWAAVVVPSGEEQRYTCHVQHEGLPKPLTLRW

SEQ ID NO: 11 - protein, 274 aa, Homo sapiens
  Cys-mut HLA-B 4402 heavy chain w/o TM domain (1)..(1)
GSHSMRYFYTAMSRPGRGEPRFITVGYVDDTLFVRFDSDATSPRKEPRAPWIEQEGPEYWDRETQISKTNTQTYRENLRTALRCYNQSEAGSHIIQRMYGCDVGPDGRLLRGYDQDAYDGKDYIALNEDLSSWTAADTCAQITQRKWEAARVAEQDRAYLEGLCVESLRRYLENGKETLQRADPPKTHVTHHPISDHEVTLRCWALGFYPAEITLTWQRDGEDQTQDTELVETRPAGDRTFQKWAAVVVPSGEEQRYTCHVQHEGLPKPLTLRW

SEQ ID NO: 12 - protein, 274 aa, Mus musculus
  Cys-mut H-2Kb heavy chain w/o TM domain (1)..(1)
GPHSLRYFVTAVSRPGLGEPRYMEVGYVDDTEFVRFDSDAENPRYEPRARWMEQEGPEYWERETQKAKGNEQSFRVDLRTLLGCYNQSKGGSHTIQVISGCEVGSDGRLLRGYQQYAYDGCDYIALNEDLKTWTAADMCALITKHKWEQAGEAERLRAYLEGTCVEWLRRYLKNGNATLLRTDSPKAHVTHHSRPEDKVTLRCWALGFYPADITLTWQLNGEELIQDMELVETRPAGDGTFQKWASVVVPLGKEQYYTCHVYHQGLPEPLTLRW

SEQ ID NO: 13 - protein, 274 aa, Mus musculus
  Cys-mut H-2Db heavy chain w/o TM domain (1)..(1)
GPHSMRYFETAVSRPGLEEPRYISVGYVDNKEFVRFDSDAENPRYEPRAPWMEQEGPEYWERETQKAKGQEQWFRVSLRNLLGCYNQSAGGSHTLQQMSGCDLGSDWRLLRGYLQFAYEGRDYIALNEDLKTWTAADMCAQITRRKWEQSGAAEHYKAYLEGECVEWLHRYLKNGNATLLRTDSPKAHVTHHPRSKGEVTLRCWALGFYPADITLTWQLNGEELTQDMELVETRPAGDGTFQKWASVVVPLGKEQNYTCRVYHEGLPEPLTLRW

SEQ ID NO: 14 - protein, 291 aa, Homo sapiens
  Cys-mut HLA-A 0201 heavy chain + Avi-tag w/o TM domain (1)..(1)
GSHSMRYFFTSVSRPGRGEPRFIAVGYVDDTQFVRFDSDAASQRMEPRAPWIEQEGPEYWDGETRKVKAHSQTHRVDLGTLRGCYNQSEAGSHTVQRMYGCDVGSDWRFLRGYHQYAYDGKDYIALKEDLRSWTAADMCAQTTKHKWEAAHVAEQLRAYLEGTCVEWLRRYLENGKETLQRTDAPKTHMTHHAVSDHEATLRCWALSFYPAEITLTWQRDGEDQTQDTELVETRPAGDGTFQKWAAVVVPSGQEQRYTCHVQHEGLPKPLTLRWASGLNDIFEAQKIEWHE

SEQ ID NO: 15 - protein, 98 aa, Homo sapiens
  Beta-2 microglobulin (B2M) (1)..(1)
QRTPKIQVYSRHPAENGKSNFLNCYVSGFHPSDIEVDLLKNGERIEKVEHSDLSFSKDWSFYLLYYTEFTPTEKDEYACRVNHVTLSQPKIVKWDRDM

SEQ ID NO: 16 - protein, 387 aa, Homo sapiens
  Cys-mut HLA-A 0201 B2M + linker + heavy chain fusion w/o TM domain (1)..(1)
QRTPKIQVYSRHPAENGKSNFLNCYVSGFHPSDIEVDLLKNGERIEKVEHSDLSFSKDWSFYLLYYTEFTPTEKDEYACRVNHVTLSQPKIVKWDRDMGGGGSGGGGSGGGGSGSHSMRYFFTSVSRPGRGEPRFIAVGYVDDTQFVRFDSDAASQRMEPRAPWIEQEGPEYWDGETRKVKAHSQTHRVDLGTLRGCYNQSEAGSHTVQRMYGCDVGSDWRFLRGYHQYAYDGKDYIALKEDLRSWTAADMCAQTTKHKWEAAHVAEQLRAYLEGTCVEWLRRYLENGKETLQRTDAPKTHMTHHAVSDHEATLRCWALSFYPAEITLTWQRDGEDQTQDTELVETRPAGDGTFQKWAAVVVPSGQEQRYTCHVQHEGLPKPLTLRW

SEQ ID NO: 17 - protein, 9 aa, Artificial sequence
  UV-labile peptide
  UV-labile peptide (1)..(1): Xaa refers to a UV sensitive amino acid, 3-amino-2-(2-nitrophenyl) propionic acid
KILGFVFXV

SEQ ID NO: 18 - protein, 9 aa, Cytomegalovirus
  CMV pp65 NLV (1)..(1)
NLVPMVATV

SEQ ID NO: 19 - protein, 9 aa, Epstein-Barr virus
  EBV BRLF1 YVL (1)..(1)
YVLDHLIVV

SEQ ID NO: 20 - protein, 9 aa, Cytomegalovirus
  CMV IE1 VLE (1)..(1)
VLEETSVML

SEQ ID NO: 21 - protein, 9 aa, Influenza virus
  FLU MP GIL (1)..(1)
GILGFVFTL

SEQ ID NO: 22 - protein, 9 aa, Epstein-Barr virus
  EBV BMF1 GLC (1)..(1)
GLCTLVAML

SEQ ID NO: 23 - protein, 9 aa, Epstein-Barr virus
  EBV LMP2 FLY (1)..(1)
FLYALALLL

SEQ ID NO: 24 - protein, 9 aa, Homo sapiens
  gp100 ITD (1)..(1)
ITDQVPFSV

SEQ ID NO: 25 - protein, 10 aa, Homo sapiens
  gp100 AML (1)..(1)
AMLGTHTMEV

SEQ ID NO: 26 - protein, 9 aa, Homo sapiens
  VANGL1 RLM (1)..(1)
RLMVAVEEA

SEQ ID NO: 27 - protein, 11 aa, Homo sapiens
  VANGL1(2) RLM (1)..(1)
RLMVAVEEAFI

SEQ ID NO: 28 - protein, 9 aa, Homo sapiens
  DYSF LLL (1)..(1)
LLLFLTIFI

SEQ ID NO: 29 - protein, 10 aa, Homo sapiens
  MEL VLY (1)..(1)
VLYRYGSFSV

SEQ ID NO: 30 - protein, 9 aa, Homo sapiens
  MEL KAS (1)..(1)
KASEKIFYV

SEQ ID NO: 31 - protein, 9 aa, Merkel Cell Polyomavirus
  MCV KLL (1)..(1)
KLLEIAPNY

SEQ ID NO: 32 - DNA, 72 bp, Artificial Sequence
  A22-B63 A-barcode
  X' 5 (1)..(1): X = Biotin-C6-
  misc_feature (26)..(31): n is a, c, g, or t
gaagttccagccagcgtcacagtttnnnnnntaatacgcctgaggtgttgggttgcggtcagcatcatttcc

SEQ ID NO: 33 - DNA, 72 bp, Artificial Sequence; identical to SEQ ID NO: 32
  A22-B64 A-barcode
  X' 5 (1)..(1): X = Biotin-C6-
  misc_feature (26)..(31): n is a, c, g, or t

SEQ ID NO: 34 - DNA, 72 bp, Artificial Sequence; identical to SEQ ID NO: 32
  A22-B65 A-barcode
  X' 5 (1)..(1): X = Biotin-C6-
  misc_feature (26)..(31): n is a, c, g, or t

SEQ ID NO: 35 - DNA, 72 bp, Artificial Sequence; identical to SEQ ID NO: 32
  A22-B71 A-barcode
  X' 5 (1)..(1): X = Biotin-C6-
  misc_feature (26)..(31): n is a, c, g, or t

SEQ ID NO: 36 - DNA, 72 bp, Artificial Sequence; identical to SEQ ID NO: 32
  A22-B75 A-barcode
  X' 5 (1)..(1): X = Biotin-C6-
  misc_feature (26)..(31): n is a, c, g, or t

SEQ ID NO: 37 - DNA, 70 bp, Artificial Sequence
  A22-B63 B-barcode
  misc_feature (24)..(29): n is a, c, g, or t
gttatcggctcgttcacactcgannnnnnccggttttataccctcgttccccgaggaaatgatgctgacc

SEQ ID NO: 38 - DNA, 70 bp, Artificial Sequence
  A22-B64 B-barcode
  misc_feature (24)..(29): n is a, c, g, or t
gttatcggctcgttcacactcgannnnnncagaactacaggctggcatggatgcggaaatgatgctgacc

SEQ ID NO: 39 - DNA, 70 bp, Artificial Sequence
  A22-B65 B-barcode
  misc_feature (24)..(29): n is a, c, g, or t
gttatcggctcgttcacactcgannnnnnattctgatgggtagaaaccgttcccggaaatgatgctgacc

SEQ ID NO: 40 - DNA, 70 bp, Artificial Sequence
  A22-B71 B-barcode
  misc_feature (24)..(29): n is a, c, g, or t
gttatcggctcgttcacactcgannnnnntttccttgttcggatcggtcgagaaggaaatgatgctgacc

SEQ ID NO: 41 - DNA, 70 bp, Artificial Sequence
  A22-B75 B-barcode
  misc_feature (24)..(29): n is a, c, g, or t
gttatcggctcgttcacactcgannnnnncatatggatttgttgcatcctgatgggaaatgatgctgacc

SEQ ID NO: 42 - DNA, 58 bp, Artificial Sequence
  Forward primer (A-Key 2OS-F1-233)
ccatctcatccctgcgtgtctccgactcagtgacaggttggaagttccagccagcgtc

SEQ ID NO: 43 - DNA, 23 bp, Artificial Sequence
  Reverse primer (P1R2)
gttatcggctcgttcacactcga